European Patent Application EP 4 365 306 A2, published May 8, 2024. Title: Methods for detecting target polynucleotides. Applicant: NunaBio Limited. The sequence listing filed with the application follows.

SEQUENCE LISTING (26 sequences)

SEQ ID NO: 1 - DNA, 10 bp, Homo sapiens
  source 1..10: mol_type = genomic DNA
gcatctttcg

SEQ ID NO: 2 - DNA, 10 bp, synthetic construct
  misc_feature 1..10: note = sequence for the heat-cool cycle extension with Tgo-Pol Z3 exo-
  source 1..10: mol_type = other DNA
cgtagaaagc

SEQ ID NO: 3 - DNA, 12 bp, synthetic construct
  misc_feature 1..12: note = sequence for heat-cool cycle extension with Tgo-Pol Z3 exo
  source 1..12: mol_type = other DNA
gaaaaaaaaaac

SEQ ID NO: 4 - DNA, 12 bp, synthetic construct
  misc_feature 1..12: note = sequence for heat-cool cycle extension with Tgo-Pol Z3 exo-
  source 1..12: mol_type = other DNA
cttttttttttg

SEQ ID NO: 5 - DNA, 10 bp, synthetic construct
  misc_feature 1..10: note = polynucleotide comprising two tandem repeats of the unit sequence
  source 1..10: mol_type = other DNA
attcgattcg

SEQ ID NO: 6 - DNA, 15 bp, synthetic construct
  misc_feature 1..15: note = polynucleotide comprising three tandem repeats of the unit sequence
  source 1..15: mol_type = other DNA
attcgattcgattcg

SEQ ID NO: 7 - DNA, 20 bp, synthetic construct
  misc_feature 1..20: note = polynucleotide comprising four tandem repeats of the unit sequence
  source 1..20: mol_type = other DNA
attcgattcgattcgattcg

SEQ ID NO: 8 - DNA, 10 bp, synthetic construct
  misc_feature 1..10: note = common unit sequences that may be tandemly repeated in the linear polynucleotide
  source 1..10: mol_type = other DNA
aaaaaaaaag

SEQ ID NO: 9 - DNA, 10 bp, synthetic construct
  misc_feature 1..10: note = common unit sequences that may be tandemly repeated in the linear polynucleotide
  source 1..10: mol_type = other DNA
actgatcagc

SEQ ID NO: 10 - DNA, 15 bp, Homo sapiens
  source 1..15: mol_type = genomic DNA
agatacattgacctt

SEQ ID NO: 11 - DNA, 15 bp, Homo sapiens
  source 1..15: mol_type = genomic DNA
gaggaccgtgttcaa

SEQ ID NO: 12 - protein, 8 aa, synthetic construct
  REGION 1..8: note = acetal protected aldehyde terminated siloxane linker (acetalpolyethyleneglycoldimethylethoxysilane)
APEGDMES

SEQ ID NO: 13 - DNA, 21 bp, synthetic construct
  misc_feature 1..21: note = CFTR-probe
  misc_feature 1: note = n is amino-C6
  source 1..21: mol_type = other DNA
ngcatctttcggcatctttcg

SEQ ID NO: 14 - DNA, 20 bp, synthetic construct
  misc_feature 1..20: note = CFTR-target
  source 1..20: mol_type = other DNA
cgaaagatgccgaaagatgc

SEQ ID NO: 15 - DNA, 10 bp, Homo sapiens
  source 1..10: mol_type = genomic DNA
gcattcgagc

SEQ ID NO: 16 - DNA, 12 bp, synthetic construct
  misc_feature 1..12: note = diagnostically important oligoseed sequence consisting of a long run of ten T-bases
  source 1..12: mol_type = other DNA
gttttttttttc

SEQ ID NO: 17 - DNA, 25 bp, synthetic construct
  misc_feature 1..25: note = BAT25-probe
  misc_feature 1: note = n is amino-c6
  source 1..25: mol_type = other DNA
ngaaaaaaaaaacgaaaaaaaaaac

SEQ ID NO: 18 - DNA, 24 bp, synthetic construct
  misc_feature 1..24: note = BAT25-target
  source 1..24: mol_type = other DNA
gttttttttttcgttttttttttc

SEQ ID NO: 19 - DNA, 20 bp, synthetic construct
  misc_feature 1..20: note = key sequence - figure 1
  source 1..20: mol_type = other DNA
gatcgatcgatcgatcgatc

SEQ ID NO: 20 - DNA, 15 bp, Homo sapiens
  source 1..15: mol_type = genomic DNA
atcatctttggtgtt

SEQ ID NO: 21 - protein, 5 aa, Homo sapiens
IIFGV

SEQ ID NO: 22 - DNA, 12 bp, Homo sapiens
  source 1..12: mol_type = genomic DNA
atcattggtgtt

SEQ ID NO: 23 - protein, 4 aa, Homo sapiens
IIGV

SEQ ID NO: 24 - DNA, 40 bp, synthetic construct
  misc_feature 1..40: note = sequence in Fig.8
  source 1..40: mol_type = other DNA
gttttttttttcgttttttttttcgttttttttttcgttt

SEQ ID NO: 25 - DNA, 11 bp, synthetic construct
  misc_feature 1..11: note = Mismatched sequences to be rehybridized with BAT25 probe - Double base mismatch
  source 1..11: mol_type = other DNA
gtttttttttc

SEQ ID NO: 26 - DNA, 10 bp, synthetic construct
  misc_feature 1..10: note = Mismatched sequences to be rehybridized with BAT25 probe - Triple base mismatch
  source 1..10: mol_type = other DNA
gttttttttc